European Patent Application EP 4 474 482 A1, published December 11, 2024. Title: Method for labeling cells. Applicant: RIKEN. The sequence listing filed with the application follows.

SEQUENCE LISTING (11 sequences)

SEQ ID NO: 1 - DNA, 15 bp, synthetic construct
  misc_feature 1..15: note = TotalSeq-A0951 PE Streptavidin
  source 1..15: mol_type = other DNA
aacctttgccactgc

SEQ ID NO: 2 - DNA, 15 bp, synthetic construct
  misc_feature 1..15: note = TotalSeq-A0952 PE Streptavidin
  source 1..15: mol_type = other DNA
gtccgactaatagct

SEQ ID NO: 3 - DNA, 15 bp, synthetic construct
  misc_feature 1..15: note = TotalSeq-A0953 PE Streptavidin
  source 1..15: mol_type = other DNA
caggttgttgtcatt

SEQ ID NO: 4 - DNA, 15 bp, synthetic construct
  misc_feature 1..15: note = TotalSeq-A0954 PE Streptavidin
  source 1..15: mol_type = other DNA
tatttccacccggtc

SEQ ID NO: 5 - DNA, 15 bp, synthetic construct
  misc_feature 1..15: note = TotalSeq-A0955 PE Streptavidin
  source 1..15: mol_type = other DNA
gttgtgagcacgaga

SEQ ID NO: 6 - DNA, 15 bp, synthetic construct
  misc_feature 1..15: note = TotalSeq-A0436 anti-Biotin Antibody
  source 1..15: mol_type = other DNA
cggtatatcaacaga

SEQ ID NO: 7 - DNA, 30 bp, synthetic construct
  misc_feature 1..30: note = 5'BDWTAv2-9G
  source 1..30: mol_type = other DNA
aagcagtggtatcaacgcagaggggggggg

SEQ ID NO: 8 - DNA, 22 bp, synthetic construct
  misc_feature 1..22: note = 5' BDWTAv2
  source 1..22: mol_type = other DNA
aagcagtggtatcaacgcagag

SEQ ID NO: 9 - DNA, 33 bp, synthetic construct
  misc_feature 1..33: note = Universal Oligo-long
  source 1..33: mol_type = other DNA
acactctttccctacacgacgctcttccgatct

SEQ ID NO: 10 - DNA, 32 bp, synthetic construct
  misc_feature 1..32: note = totalseq-ADT-oligo1
  source 1..32: mol_type = other DNA
tgctcttccgatcttggcacccgagaattcca

SEQ ID NO: 11 - DNA, 37 bp, synthetic construct
  misc_feature 1..37: note = totalseq-ADT-oligo2
  source 1..37: mol_type = other DNA
gtgactggagttcagacgtgtgctcttccgatcttgg